European Patent Application EP 4 455 664 A1, published October 30, 2024. Title: Composition comprising TAF10 inhibitor for prevention or treatment of colorectal cancer. Applicant: Korea Advanced Institute of Science and Technology. Application KR. The sequence listing filed with the application follows.

SEQUENCE LISTING (33 sequences)

SEQ ID NO: 1 - RNA, 19 nt, synthetic construct
  source 1..19: mol_type = other RNA; note = siTAF10-SENSE
gtgaagaagccgcactact

SEQ ID NO: 2 - RNA, 19 nt, synthetic construct
  source 1..19: mol_type = other RNA; note = siTAF10-ANTISENSE
agtagtgcggcttcttcac

SEQ ID NO: 3 - RNA, 23 nt, synthetic construct
  source 1..23: mol_type = other RNA; note = siNPM1-SENSE
gaagcagaggcaatgaattacga

SEQ ID NO: 4 - RNA, 23 nt, synthetic construct
  source 1..23: mol_type = other RNA; note = siNPM1-ANTISENSE
tcgtaattcattgcctctgcttc

SEQ ID NO: 5 - RNA, 19 nt, synthetic construct
  source 1..19: mol_type = other RNA; note = siZNHIT1-SENSE
gagactgcctcagtttgat

SEQ ID NO: 6 - RNA, 19 nt, synthetic construct
  source 1..19: mol_type = other RNA; note = siZNHIT1-ANTISENSE
atcaaactgaggcagtctc

SEQ ID NO: 7 - RNA, 21 nt, synthetic construct
  source 1..21: mol_type = other RNA; note = shTAF10
ccgcaagtacactctaaccat

SEQ ID NO: 8 - DNA, 20 bp, synthetic construct
  source 1..20: mol_type = other DNA; note = TAF10 forward primer
ccacgcataattcggctcat

SEQ ID NO: 9 - DNA, 21 bp, synthetic construct
  source 1..21: mol_type = other DNA; note = TAF10 reverse primer
cctccatggttagggtgtact

SEQ ID NO: 10 - DNA, 25 bp, synthetic construct
  source 1..25: mol_type = other DNA; note = GAPDH forward primer
tgatgacatcaagaaggtggtgaag

SEQ ID NO: 11 - DNA, 23 bp, synthetic construct
  source 1..23: mol_type = other DNA; note = GAPDH reverse primer
tccttggaggccatgtgggccat

SEQ ID NO: 12 - DNA, 22 bp, synthetic construct
  source 1..22: mol_type = other DNA; note = MKI67 forward primer
gaaagagtggcaacctgccttc

SEQ ID NO: 13 - DNA, 24 bp, synthetic construct
  source 1..24: mol_type = other DNA; note = MKI67 reverse primer
gcaccaagttttactacatctgcc

SEQ ID NO: 14 - DNA, 24 bp, synthetic construct
  source 1..24: mol_type = other DNA; note = PCNA forward primer
caagtaatgtcgataaagaggagg

SEQ ID NO: 15 - DNA, 22 bp, synthetic construct
  source 1..22: mol_type = other DNA; note = PCNA reverse primer
gtgtcaccgttgaagagagtgg

SEQ ID NO: 16 - DNA, 22 bp, synthetic construct
  source 1..22: mol_type = other DNA; note = MCM7 forward primer
gccaagtctcagctcctgtcat

SEQ ID NO: 17 - DNA, 23 bp, synthetic construct
  source 1..23: mol_type = other DNA; note = MCM7 reverse primer
cctctaaggtcagttctccactc

SEQ ID NO: 18 - DNA, 22 bp, synthetic construct
  source 1..22: mol_type = other DNA; note = TP53 forward primer
cctcagcatcttatccgagtgg

SEQ ID NO: 19 - DNA, 22 bp, synthetic construct
  source 1..22: mol_type = other DNA; note = TP53 reverse primer
tggatggtggtacagtcagagc

SEQ ID NO: 20 - DNA, 22 bp, synthetic construct
  source 1..22: mol_type = other DNA; note = CDKN1A forward primer
aggtggacctggagactctcag

SEQ ID NO: 21 - DNA, 22 bp, synthetic construct
  source 1..22: mol_type = other DNA; note = CDKN1A reverse primer
tcctcttggagaagatcagccg

SEQ ID NO: 22 - DNA, 20 bp, synthetic construct
  source 1..20: mol_type = other DNA; note = CXCL8 forward primer
gtgcagttttgccaaggagt

SEQ ID NO: 23 - DNA, 20 bp, synthetic construct
  source 1..20: mol_type = other DNA; note = CXCL8 reverse primer
ctctgcacccagttttcctt

SEQ ID NO: 24 - DNA, 22 bp, synthetic construct
  source 1..22: mol_type = other DNA; note = CTNNB1 forward primer
cacaagcagagtgctgaaggtg

SEQ ID NO: 25 - DNA, 23 bp, synthetic construct
  source 1..23: mol_type = other DNA; note = CTNNB1 reverse primer
gattcctgagagtccaaagacag

SEQ ID NO: 26 - DNA, 22 bp, synthetic construct
  source 1..22: mol_type = other DNA; note = CCND1 forward primer
tctacaccgacaactccatccg

SEQ ID NO: 27 - DNA, 23 bp, synthetic construct
  source 1..23: mol_type = other DNA; note = CCND1 reverse primer
tctggcattttggagaggaagtg

SEQ ID NO: 28 - DNA, 19 bp, synthetic construct
  source 1..19: mol_type = other DNA; note = TCF7 forward primer
gacatcagccagaagcaag

SEQ ID NO: 29 - DNA, 20 bp, synthetic construct
  source 1..20: mol_type = other DNA; note = TCF7 reverse primer
caccagaacctagcatcaag

SEQ ID NO: 30 - DNA, 21 bp, synthetic construct
  source 1..21: mol_type = other DNA; note = AXIN2 forward primer
gaggagcgatcctgttaatcc

SEQ ID NO: 31 - DNA, 21 bp, synthetic construct
  source 1..21: mol_type = other DNA; note = AXIN2reverse primer
ggttctcgggaaatgaggtag

SEQ ID NO: 32 - DNA, 20 bp, synthetic construct
  source 1..20: mol_type = other DNA; note = KRT19 forward primer
gcgagctagaggtgaagatc

SEQ ID NO: 33 - DNA, 19 bp, synthetic construct
  source 1..19: mol_type = other DNA; note = KRT19 reverse primer
cggaagtcatctgcagcca